European Patent Application EP 4 521 115 A2, published March 12, 2025. Title: METHODS OF DETECTING METHYLATED CpG. Applicant: Ramot at Tel-Aviv University Ltd. EBENSTEIN, Yuval ZIRKIN, Shahar MICHAELI-HOCH, Yael GILAT, Noa FELDSTEIN, Orit BEN-MOSHE, Adaya. The sequence listing filed with the application follows.

SEQUENCE LISTING (10 sequences)

SEQ ID NO: 1 - DNA, 25 bp, Artificial sequence
  Adapter 1 nucleic acid sequence
gtctagggaacataggatcaggact

SEQ ID NO: 2 - DNA, 21 bp, Artificial sequence
  Single strand DNA oligonucleotide
gtctagggaacataggatcag

SEQ ID NO: 3 - DNA, 29 bp, Artificial sequence
  Adapter 2 nucleic acid sequence
  misc_feature (1)..(1): 5' phosphate group conjugated
gtcctgatcctattaatgactacaacttg

SEQ ID NO: 4 - DNA, 21 bp, Artificial sequence
  Single strand DNA oligonucleotide
caagttgtagtcattaatagg

SEQ ID NO: 5 - DNA, 25 bp, Artificial Sequence
  Adapter 3 nucleic acid sequence
gtctagggaacataggatcaggact

SEQ ID NO: 6 - DNA, 21 bp, Artificial Sequence
  Single strand DNA oligonucleotide
gtctagggaacataggatgtc

SEQ ID NO: 7 - DNA, 25 bp, Artificial Sequence
  Adapter 4 nucleic acid sequence
  misc_feature (1)..(1): 5' phosphate group conjugated
ggagactattggtgactacaacttg

SEQ ID NO: 8 - DNA, 22 bp, Artificial Sequence
  Single strand DNA oligonucleotide
caagttgtagtcaccaatagtc

SEQ ID NO: 9 - DNA, 32 bp, Artificial Sequence
  Single strand DNA oligonucleotide
gtttggtaatttatttagagaagtaaaatgat

SEQ ID NO: 10 - DNA, 28 bp, Artificial Sequence
  Single strand DNA oligonucleotide
tacaaatcccacaaataaaaaaaatact